European Patent Application EP 4 793 277 A1, published August 19, 2026. Title: 一类羧酸类化合物及其制备方法和应用. Applicant: 上海宇道生物技术有限公司. Application CN. The sequence listing filed with the application follows.

SEQUENCE LISTING (1 sequence)

SEQ ID NO: 1 - DNA, 26 bp, synthetic construct
  source 1..26: mol_type = other DNA
attaggcatgtctaggcatgtctagg